European Patent Specification EP 3 727 369 B1, published December 17, 2025. Title: THERANOSTIC TEST FOR ANTIFUNGAL TREATMENT OF INFLAMMATORY DISEASES. Applicant: Cornell University. The sequence listing filed with the application follows.

SEQUENCE LISTING (31 sequences)

SEQ ID NO: 1 - DNA, 51 bp, Homo sapiens
caggcaacaatggctaaatgcaaccatctcagtcacactgagggccagcct

SEQ ID NO: 2 - DNA, 51 bp, Homo sapiens
ttaagcgtctccaggaaaatcataatgttgtagggtgtccagaagaggaaa

SEQ ID NO: 3 - DNA, 51 bp, Homo sapiens
ctgaatcagtgacagaaaactttgattacgatgatttggctgaggcctgtt

SEQ ID NO: 4 - DNA, 20 bp, Artificial Sequence
  Primer
cttctggacaccctacaacg

SEQ ID NO: 5 - DNA, 23 bp, Artificial Sequence
  Primer
cctcttctggacaccctacaaca

SEQ ID NO: 6 - DNA, 27 bp, Artificial Sequence
  Primer
gagcttaagygtctccaggaaaatcat

SEQ ID NO: 7 - DNA, 21 bp, Artificial Sequence
  Primer
ggccctcagtgtgactgagac

SEQ ID NO: 8 - DNA, 21 bp, Artificial Sequence
  Primer
ggccctcagtgtgactgagat

SEQ ID NO: 9 - DNA, 25 bp, Artificial Sequence
  Primer
gagaggattcaggcaacaatggcta

SEQ ID NO: 10 - protein, 17 aa, Gallus gallus
ISQAVHAAHAEINEAGR

SEQ ID NO: 11 - DNA, 95 bp, Artificial Sequence
  Primer
ccggggatccgaatctttgaaaatttctcaagctgttcacgctgctcacgctgaaattaacgaagctggtagagaagttgttggtagatctggcc

SEQ ID NO: 12 - DNA, 94 bp, Artificial Sequence
  Primer
gccagatctaccaacaacttctctaccagcttcgttaatttcagcgtgagcagcgtgaacagcttgagaaattttcaaagattcggatccccgg

SEQ ID NO: 13 - DNA, 42 bp, Artificial Sequence
  Primer
ggccggatccgcggccgcatgagtaaaggagaagaacttttc

SEQ ID NO: 14 - DNA, 37 bp, Artificial Sequence
  Primer
ggccagatcttttgtatagttcatccatgccatgtgt

SEQ ID NO: 15 - DNA, 43 bp, Artificial Sequence
  Primer
atataaatactcgagaaagatgagtaagggagaagaacttttc

SEQ ID NO: 16 - DNA, 34 bp, Artificial Sequence
  Primer
atttagatctttacatgatgcggccctcctgcag

SEQ ID NO: 17 - DNA, 22 bp, Artificial Sequence
  Primer
cttggtcatttagaggaagtaa

SEQ ID NO: 18 - DNA, 20 bp, Artificial Sequence
  Primer
gctgcgttcttcatcgatgc

SEQ ID NO: 19 - DNA, 20 bp, Artificial Sequence
  Primer
agagtttgatcmtggctcag

SEQ ID NO: 20 - DNA, 15 bp, Artificial Sequence
  Primer
ctgctgcctyccgta

SEQ ID NO: 21 - DNA, 33 bp, Artificial Sequence
  Primer
tcgtcggcagcgtcagatgtgtataagagacag

SEQ ID NO: 22 - DNA, 34 bp, Artificial Sequence
  Primer
gtctcgtgggctcggagatgtgtataagagacag

SEQ ID NO: 23 - DNA, 21 bp, Artificial Sequence
  Primer
actcctacgggaggcagcagt

SEQ ID NO: 24 - DNA, 18 bp, Artificial Sequence
  Primer
attaccgcggctgctggc

SEQ ID NO: 25 - DNA, 20 bp, Artificial Sequence
  Primer
attggagggcaagtctggtg

SEQ ID NO: 26 - DNA, 20 bp, Artificial Sequence
  Primer
ccgatccctagtcggcatag

SEQ ID NO: 27 - DNA, 18 bp, Artificial Sequence
  Primer
cctgtttgagcgtcgttt

SEQ ID NO: 28 - DNA, 18 bp, Artificial Sequence
  Primer
tcctccgcttattgatat

SEQ ID NO: 29 - DNA, 22 bp, Artificial Sequence
  Primer
ggaagtaaaagtcgtaacaagg

SEQ ID NO: 30 - DNA, 23 bp, Artificial Sequence
  Primer
cgttactrrggcaatccctgttg

SEQ ID NO: 31 - DNA, 18 bp, Artificial Sequence
  Primer
gcrcggaaracgcttctc